European Patent Application EP 4 292 659 A2, published December 20, 2023. Title: ANTIBODIES THAT NEUTRALIZE HEPATITIS B VIRUS AND USES THEREOF. Applicant: Humabs BioMed SA. Application EP, filed August 25, 2023. The sequence listing filed with the application follows.

SEQUENCE LISTING (139 sequences)

SEQ ID NO: 1 - protein, 11 aa, Hepatitis B virus
XXXTCXXXAXG

SEQ ID NO: 2 - protein, 11 aa, Hepatitis B virus
  VARIANT 1: note = Xaa = P, T or S,
  VARIANT 2: note = Xaa = C or S,
  VARIANT 3: note = Xaa = R, K, D or I,
  VARIANT 6: note = Xaa = M or T
  VARIANT 7: note = Xaa = T, A or I
  VARIANT 8: note = Xaa = T, P or L
  VARIANT 10: note = Xaa = Q, H or L.
XXXTCXXXAXG

SEQ ID NO: 3 - protein, 226 aa, Hepatitis B virus
  REGION 1..226: note = S domain of HBsAg (GenBank acc. no. J02203)
MENITSGFLGPLLVLQAGFFLLTRILTIPQSLDSWWTSLNFLGGTTVCLGQNSQSPTSNHSPTSCPPTCPGYRWMCLRRFIIFLFILLLCLIFLLVLLDYQGMLPVCPLIPGSSTTSTGPCRTCMTTAQGTSMYPSCCCTKPSDGNCTCIPIPSSWAFGKFLWEWASARFSWLSLLVPFVQWFVGLSPTVWLSVIWMMWYWGPSLYSILSPFLPLLPIFFCLWVYI

SEQ ID NO: 4 - protein, 226 aa, Hepatitis B virus
  REGION 1..226: note = S domain of HBsAg (GenBank acc. no. FJ899792)
MENVTSGFLGPLLVLQAGFFLLTRILTIPQSLDSWWTSLNFLGGTTVCLGQNSQSPTSNHSPTSCPPTCPGYRWMCLRRFIIFLFILLLCLIFLLVLLDYQGMLPVCPLIPGSSTTGTGPCRTCTTPAQGTSMYPSCCCTKPSDGNCTCIPIPSSWAFGKFLWEWASARFSWLSLLVPFVQWFVGLSPTVWLSVIWMMWYWGPSLYSTLSPFLPLLPIFFCLWVYI

SEQ ID NO: 5 - protein, 72 aa, Hepatitis B virus
  REGION 1..72: note = J02203 (D, ayw3)
QGMLPVCPLIPGSSTTSTGPCRTCMTTAQGTSMYPSCCCTKPSDGNCTCIPIPSSWAFGKFLWEWASARFSW

SEQ ID NO: 6 - protein, 72 aa, Hepatitis B virus
  REGION 1..72: note = FJ899792 (D, adw2)
QGMLPVCPLIPGSSTTGTGPCRTCTTPAQGTSMYPSCCCTKPSDGNCTCIPIPSSWAFGKFLWEWASARFSW

SEQ ID NO: 7 - protein, 72 aa, Hepatitis B virus
  REGION 1..72: note = AM282986 (A)
QGMLPVCPLIPGTTTTSTGPCKTCTTPAQGNSMFPSCCCTKPSDGNCTCIPIPSSWAFAKYLWEWASVRFSW

SEQ ID NO: 8 - protein, 72 aa, Hepatitis B virus
  REGION 1..72: note = D23678 (B1)
QGMLPVCPLIPGSSTTSTGPCKTCTTPAQGTSMFPSCCCTKPTDGNCTCIPIPSSWAFAKYLWEWASVRFSW

SEQ ID NO: 9 - protein, 72 aa, Hepatitis B virus
  REGION 1..72: note = AB117758 (C1)
QGMLPVCPLLPGTSTTSTGPCKTCTIPAQGTSMFPSCCCTKPSDGNCTCIPIPSSWAFARFLWEWASVRFSW

SEQ ID NO: 10 - protein, 72 aa, Hepatitis B virus
  REGION 1..72: note = AB205192 (E)
QGMLPVCPLIPGSSTTSTGPCRTCTTLAQGTSMFPSCCCSKPSDGNCTCIPIPSSWAFGKFLWEWASARFSW

SEQ ID NO: 11 - protein, 72 aa, Hepatitis B virus
  REGION 1..72: note = X69798 (F4)
QGMLPVCPLLPGSTTTSTGPCKTCTTLAQGTSMFPSCCCSKPSDGNCTCIPIPSSWALGKYLWEWASARFSW

SEQ ID NO: 12 - protein, 72 aa, Hepatitis B virus
  REGION 1..72: note = AF160501 (G)
QGMLPVCPLIPGSSTTSTGPCKTCTTPAQGNSMYPSCCCTKPSDGNCTCIPIPSSWAFAKYLWEWASVRFSW

SEQ ID NO: 13 - protein, 72 aa, Hepatitis B virus
  REGION 1..72: note = AY090454 (H)
QGMLPVCPLLPGSTTTSTGPCKTCTTLAQGTSMFPSCCCTKPSDGNCTCIPIPSSWAFGKYLWEWASARFSW

SEQ ID NO: 14 - protein, 72 aa, Hepatitis B virus
  REGION 1..72: note = AF241409 (I)
QGMLPVCPLIPGSSTTSTGPCKTCTTPAQGNSMYPSCCCTKPSDGNCTCIPIPSSWAFAKYLWEWASARFSW

SEQ ID NO: 15 - protein, 72 aa, Hepatitis B virus
  REGION 1..72: note = AB486012 (J)
QGMLPVCPLLPGSTTTSTGPCRTCTITAQGTSMFPSCCCTKPSDGNCTCIPIPSSWAFAKFLWEWASVRFSW

SEQ ID NO: 16 - protein, 73 aa, Hepatitis B virus
  REGION 1..73: note = HBsAg Y100C/P120T
CQGMLPVCPLIPGSSTTGTGTCRTCTTPAQGTSMYPSCCCTKPSDGNCTCIPIPSSWAFGKFLWEWASARFSW

SEQ ID NO: 17 - protein, 72 aa, Hepatitis B virus
  REGION 1..72: note = HBsAg P120T
QGMLPVCPLIPGSSTTGTGTCRTCTTPAQGTSMYPSCCCTKPSDGNCTCIPIPSSWAFGKFLWEWASARFSW

SEQ ID NO: 18 - protein, 72 aa, Hepatitis B virus
  REGION 1..72: note = HBsAg P120T/S143L
QGMLPVCPLIPGSSTTGTGTCRTCTTPAQGTSMYPSCCCTKPLDGNCTCIPIPSSWAFGKFLWEWASARFSW

SEQ ID NO: 19 - protein, 72 aa, Hepatitis B virus
  REGION 1..72: note = HBsAg C121S
QGMLPVCPLIPGSSTTGTGPSRTCTTPAQGTSMYPSCCCTKPSDGNCTCIPIPSSWAFGKFLWEWASARFSW

SEQ ID NO: 20 - protein, 72 aa, Hepatitis B virus
  REGION 1..72: note = HBsAg R122D
QGMLPVCPLIPGSSTTGTGPCDTCTTPAQGTSMYPSCCCTKPSDGNCTCIPIPSSWAFGKFLWEWASARFSW

SEQ ID NO: 21 - protein, 72 aa, Hepatitis B virus
  REGION 1..72: note = HBsAg R122I
QGMLPVCPLIPGSSTTGTGPCITCTTPAQGTSMYPSCCCTKPSDGNCTCIPIPSSWAFGKFLWEWASARFSW

SEQ ID NO: 22 - protein, 72 aa, Hepatitis B virus
  REGION 1..72: note = HBsAg T123N
QGMLPVCPLIPGSSTTGTGPCRNCTTPAQGTSMYPSCCCTKPSDGNCTCIPIPSSWAFGKFLWEWASARFSW

SEQ ID NO: 23 - protein, 72 aa, Hepatitis B virus
  REGION 1..72: note = HBsAg Q129H
QGMLPVCPLIPGSSTTGTGPCRTCTTPAHGTSMYPSCCCTKPSDGNCTCIPIPSSWAFGKFLWEWASARFSW

SEQ ID NO: 24 - protein, 72 aa, Hepatitis B virus
  REGION 1..72: note = HBsAg Q129L
QGMLPVCPLIPGSSTTGTGPCRTCTTPALGTSMYPSCCCTKPSDGNCTCIPIPSSWAFGKFLWEWASARFSW

SEQ ID NO: 25 - protein, 72 aa, Hepatitis B virus
  REGION 1..72: note = HBsAg M133H
QGMLPVCPLIPGSSTTGTGPCRTCTTPAQGTSHYPSCCCTKPSDGNCTCIPIPSSWAFGKFLWEWASARFSW

SEQ ID NO: 26 - protein, 72 aa, Hepatitis B virus
  REGION 1..72: note = HBsAg M133L
QGMLPVCPLIPGSSTTGTGPCRTCTTPAQGTSLYPSCCCTKPSDGNCTCIPIPSSWAFGKFLWEWASARFSW

SEQ ID NO: 27 - protein, 72 aa, Hepatitis B virus
  REGION 1..72: note = HBsAg M133T
QGMLPVCPLIPGSSTTGTGPCRTCTTPAQGTSTYPSCCCTKPSDGNCTCIPIPSSWAFGKFLWEWASARFSW

SEQ ID NO: 28 - protein, 72 aa, Hepatitis B virus
  REGION 1..72: note = HBsAg K141E
QGMLPVCPLIPGSSTTGTGPCRTCTTPAQGTSMYPSCCCTEPSDGNCTCIPIPSSWAFGKFLWEWASARFSW

SEQ ID NO: 29 - protein, 72 aa, Hepatitis B virus
  REGION 1..72: note = HBsAg P142S
QGMLPVCPLIPGSSTTGTGPCRTCTTPAQGTSMYPSCCCTKSSDGNCTCIPIPSSWAFGKFLWEWASARFSW

SEQ ID NO: 30 - protein, 72 aa, Hepatitis B virus
  REGION 1..72: note = HBsAg S143K
QGMLPVCPLIPGSSTTGTGPCRTCTTPAQGTSMYPSCCCTKPKDGNCTCIPIPSSWAFGKFLWEWASARFSW

SEQ ID NO: 31 - protein, 72 aa, Hepatitis B virus
  REGION 1..72: note = HBsAg D144A
QGMLPVCPLIPGSSTTGTGPCRTCTTPAQGTSMYPSCCCTKPSAGNCTCIPIPSSWAFGKFLWEWASARFSW

SEQ ID NO: 32 - protein, 72 aa, Hepatitis B virus
  REGION 1..72: note = HBsAg G145R
QGMLPVCPLIPGSSTTGTGPCRTCTTPAQGTSMYPSCCCTKPSDRNCTCIPIPSSWAFGKFLWEWASARFSW

SEQ ID NO: 33 - protein, 72 aa, Hepatitis B virus
  REGION 1..72: note = HBsAg N146A
QGMLPVCPLIPGSSTTGTGPCRTCTTPAQGTSMYPSCCCTKPSDGACTCIPIPSSWAFGKFLWEWASARFSW

SEQ ID NO: 34 - protein, 8 aa, synthetic construct
  REGION 1..8: note = Synthetic sequence HBC34 CDRH1
GRIFRSFY

SEQ ID NO: 35 - protein, 7 aa, synthetic construct
  REGION 1..7: note = Synthetic sequence HBC34 CDRH2
NQDGSEK

SEQ ID NO: 36 - protein, 12 aa, synthetic construct
  REGION 1..12: note = Synthetic sequence HBC34 CDRH3
AAWSGNSGGMDV

SEQ ID NO: 37 - protein, 6 aa, synthetic construct
  REGION 1..6: note = Synthetic sequence HBC34 CDRL1
KLGNKN

SEQ ID NO: 38 - skipped

SEQ ID NO: 39 - protein, 9 aa, synthetic construct
  REGION 1..9: note = Synthetic sequence HBC34 CDRL2 long
VIYEVKYRP

SEQ ID NO: 40 - protein, 9 aa, synthetic construct
  REGION 1..9: note = Synthetic sequence HBC34 CDRL3
QTWDSTTVV

SEQ ID NO: 41 - protein, 119 aa, synthetic construct
  REGION 1..119: note = Synthetic sequence HBC34, HBC34-V7, HBC34-V34, HBC34-V35 VH
ELQLVESGGGWVQPGGSQRLSCAASGRIFRSFYMSWVRQAPGKGLEWVATINQDGSEKLYVDSVKGRFTISRDNAKNSLFLQMNNLRVEDTAVYYCAAWSGNSGGMDVWGQGTTVSVSS

SEQ ID NO: 42 - protein, 106 aa, synthetic construct
  REGION 1..106: note = Synthetic sequence HBC34 VL
SYELTQPPSVSVSPGQTVSIPCSGDKLGNKNVCWFQHKPGQSPVLVIYEVKYRPSGIPERFSGSNSGNTATLTISGTQAMDEAAYFCQTWDSTTVVFGGGTRLTVL

SEQ ID NO: 43 - DNA, 24 bp, synthetic construct
  misc_feature 1..24: note = Synthetic sequence HBC34 CDRH1
  source 1..24: mol_type = other DNA
ggacgcatctttagaagtttttac

SEQ ID NO: 44 - DNA, 24 bp, synthetic construct
  misc_feature 1..24: note = Synthetic sequence HBC34 CDRH2
  source 1..24: mol_type = other DNA
ataaaccaagatggaagtgagaaa

SEQ ID NO: 45 - DNA, 36 bp, synthetic construct
  misc_feature 1..36: note = Synthetic sequence HBC34 CDRH3
  source 1..36: mol_type = other DNA
gcggcttggagcggcaatagtgggggtatggacgtc

SEQ ID NO: 46 - DNA, 18 bp, synthetic construct
  misc_feature 1..18: note = Synthetic sequence HBC34 CDRL1
  source 1..18: mol_type = other DNA
aaattggggaataaaaat

SEQ ID NO: 47 - skipped

SEQ ID NO: 48 - DNA, 27 bp, synthetic construct
  misc_feature 1..27: note = Synthetic sequence HBC34 CDRL2 long
  source 1..27: mol_type = other DNA
gtcatctatgaggttaaataccgcccc

SEQ ID NO: 49 - DNA, 27 bp, synthetic construct
  misc_feature 1..27: note = Synthetic sequence HBC34 CDRL3
  source 1..27: mol_type = other DNA
cagacgtgggacagcaccactgtggtg

SEQ ID NO: 50 - DNA, 357 bp, synthetic construct
  misc_feature 1..357: note = Synthetic sequence HBC34 VH
  source 1..357: mol_type = other DNA
gaactgcagctggtggagtctgggggaggctgggtccagccgggggggtcccagagactgtcctgtgcagcctctggacgcatctttagaagtttttacatgagctgggtccgccaggccccagggaaggggctggagtgggtggccactataaaccaagatggaagtgagaaattatatgtggactctgtgaagggccgattcaccatctccagagacaacgccaagaactcactatttctgcaaatgaacaacctgagagtcgaggacacggccgtttattactgcgcggcttggagcggcaatagtgggggtatggacgtctggggccaggggaccacggtctccgtctcctca

SEQ ID NO: 51 - DNA, 318 bp, synthetic construct
  misc_feature 1..318: note = Synthetic sequence HBC34 VL
  source 1..318: mol_type = other DNA
tcctatgagctgactcagccaccctcagtgtccgtgtccccaggacagacagtcagcatcccctgctctggagataaattggggaataaaaatgtttgctggtttcagcataagccaggccagtcccctgtgttggtcatctatgaggttaaataccgcccctcggggattcctgagcgattctctggctccaactctgggaacacagccactctgaccatcagcgggacccaggctatggatgaggctgcctatttctgtcagacgtgggacagcaccactgtggtgttcggcggagggaccaggctgaccgtccta

SEQ ID NO: 52 - protein, 33 aa, Hepatitis B virus
XGSSTTSTGPCRTCMTXPSDGNATAIPIPSSWX

SEQ ID NO: 53 - protein, 15 aa, Hepatitis B virus
TSTGPCRTCMTTAQG

SEQ ID NO: 54 - protein, 26 aa, Hepatitis B virus
GMLPVCPLIPGSSTTSTGPCRTCMTT

SEQ ID NO: 55 - protein, 33 aa, Hepatitis B virus
XSMYPSASATKPSDGNXTGPCRTCMTTAQGTSX

SEQ ID NO: 56 - protein, 11 aa, Hepatitis B virus
  REGION 1..11: note = amino acids 120 - 130 of the S domain of HBsAg (HBV-D J02203)
PCRTCMTTAQG

SEQ ID NO: 57 - protein, 11 aa, Hepatitis B virus
  VARIANT 3: note = Xaa = R or K
  VARIANT 6: note = Xaa = M or T
  VARIANT 7: note = Xaa = T or I
  VARIANT 8: note = Xaa = T, P or L
PCXTCXXXAQG

SEQ ID NO: 58 - protein, 9 aa, synthetic construct
  REGION 1..9: note = Synthetic sequence HBC34-V7 CDRL3 and HBC34-V23 CDRL3
QTFDSTTVV

SEQ ID NO: 59 - protein, 106 aa, synthetic construct
  REGION 1..106: note = Synthetic sequence HBC34-V7 VL
SYELTQPPSVSVSPGQTVSIPCSGDKLGNKNVCWFQHKPGQSPVLVIYEVKYRPSGIPERFSGSNSGNTATLTISGTQAMDEAAYFCQTFDSTTVVFGGGTRLTVL

SEQ ID NO: 60 - DNA, 18 bp, synthetic construct
  misc_feature 1..18: note = Synthetic sequence HBC34v7 CDRL1 and HBC-V23 CDRL1
  source 1..18: mol_type = other DNA
aagctggggaacaaaaat

SEQ ID NO: 61 - skipped

SEQ ID NO: 62 - DNA, 27 bp, synthetic construct
  misc_feature 1..27: note = Synthetic sequence HBC34-V7 CDRL2 long and CDRL2 HBC34-V23 long
  source 1..27: mol_type = other DNA
gtcatctacgaggtgaaatatcggcct

SEQ ID NO: 63 - DNA, 27 bp, synthetic construct
  misc_feature 1..27: note = Synthetic sequence CDRL3 HBC34-V7 and CDRL3 HBC34-V23
  source 1..27: mol_type = other DNA
cagacattcgattccaccacagtggtc

SEQ ID NO: 64 - DNA, 318 bp, synthetic construct
  misc_feature 1..318: note = Synthetic sequence HBC34-V7, HBC34-V34, and HBC34-V35 VL
  source 1..318: mol_type = other DNA
tcttacgagctgacacagccacctagcgtgtccgtctctccaggacagaccgtgtccatcccttgctctggcgacaagctggggaacaaaaatgtctgttggttccagcacaagccagggcagagtcccgtgctggtcatctacgaggtgaaatatcggccttcaggaattccagaacggttcagcggatcaaacagcggcaatactgcaaccctgacaattagcgggacccaggccatggacgaagccgcttatttctgccagacattcgattccaccacagtggtctttggcgggggaactaggctgaccgtgctg

SEQ ID NO: 65 - protein, 106 aa, synthetic construct
  REGION 1..106: note = Synthetic sequence HBC34-V23 VL
SYELTQPPSVSVSPGQTASITCSGDKLGNKNACWYQQKPGQSPVLVIYEVKYRPSGIPERFSGSNSGNTATLTISGTQAMDEADYYCQTFDSTTVVFGGGTKLTVL

SEQ ID NO: 66 - protein, 8 aa, synthetic construct
  REGION 1..8: note = Synthetic sequence HBC34wt CDRH2
INQDGSEK

SEQ ID NO: 67 - protein, 119 aa, synthetic construct
  REGION 1..119: note = Synthetic sequence HBC34-V31, HBC34-V32 and HBC34-V33 VH
EVQLVESGGGLVQPGGSLRLSCAASGRIFRSFYMSWVRQAPGKGLEWVANINQDGSEKLYVDSVKGRFTISRDNAKNSLFLQMNNLRVEDTAVYYCAAWSGNSGGMDVWGQGTTVTVSS

SEQ ID NO: 68 - DNA, 357 bp, synthetic construct
  misc_feature 1..357: note = Synthetic sequence HBC34-V31, HBC34-V32 and HBC34-V33 VH
  source 1..357: mol_type = other DNA
gaggtgcagctggtggaatccggcgggggactggtgcagcctggcggctcactgagactgagctgtgcagcttctggaagaatcttcagatctttttacatgagttgggtgagacaggctcctgggaagggactggagtgggtcgcaaacatcaatcaggacggatcagaaaagctgtatgtggatagcgtcaaaggcaggttcactatttcccgcgacaacgccaaaaattctctgtttctgcagatgaacaatctgcgggtggaggataccgctgtctactattgtgcagcctggtctggcaacagtggaggcatggacgtgtggggacagggaaccacagtgacagtcagctcc

SEQ ID NO: 69 - DNA, 318 bp, synthetic construct
  misc_feature 1..318: note = Synthetic sequence HBC34v23 VL
  source 1..318: mol_type = other DNA
tcttacgagctgacacagccccctagcgtgtccgtctctccaggccagacagcatccatcacttgctctggcgacaagctggggaacaaaaatgcctgttggtatcagcagaagccagggcagagtcccgtgctggtcatctacgaggtgaaatatcggccttcaggaattccagaaagattcagtggatcaaacagcggcaatactgctaccctgacaattagcgggacccaggccatggacgaagctgattactattgccagacattcgattccaccacagtggtctttggcgggggaactaagctgaccgtgctg

SEQ ID NO: 70 - DNA, 357 bp, synthetic construct
  misc_feature 1..357: note = Synthetic sequence HBC34 wt VH codon optimized
  source 1..357: mol_type = other DNA
gaactgcagctggtcgaatcaggaggagggtgggtccagcccggagggagccagagactgtcttgtgccgcatcagggaggatcttcaggagcttctacatgtcctgggtgcgccaggcaccaggcaagggactggagtgggtcgccaccatcaaccaggacggatctgaaaagctgtatgtggatagtgtcaaaggccggttcacaattagcagagacaacgctaaaaattctctgtttctgcagatgaacaatctgcgagtggaggataccgccgtctactattgcgccgcttggtctggcaacagcggcgggatggatgtctgggggcagggcacaacagtgagcgtctcttcc

SEQ ID NO: 71 - DNA, 318 bp, synthetic construct
  misc_feature 1..318: note = Synthetic sequence HBC34 wt VL codon optimized
  source 1..318: mol_type = other DNA
tcatacgaactgactcagcctccctccgtctccgtctcacctggacagaccgtctcaatcccctgctccggcgataaactgggcaacaagaacgtgtgctggttccagcacaaacccggacagagtcctgtgctggtcatctacgaggtcaagtatcggccaagcggcattcccgaaagattcagcggctccaactctgggaataccgcaacactgactatctctggaacccaggcaatggacgaggcagcttacttttgccagacttgggattcaactactgtcgtgttcggcggcggaactagactgactgtcctg

SEQ ID NO: 72 - DNA, 24 bp, synthetic construct
  misc_feature 1..24: note = Synthetic sequence HBC34 wt CDRH1 codon optimized
  source 1..24: mol_type = other DNA
gggaggatcttcaggagcttctac

SEQ ID NO: 73 - DNA, 24 bp, synthetic construct
  misc_feature 1..24: note = Synthetic sequence HBC34 wt CDRH2 codon optimized
  source 1..24: mol_type = other DNA
atcaaccaggacggatctgaaaag

SEQ ID NO: 74 - DNA, 36 bp, synthetic construct
  misc_feature 1..36: note = Synthetic sequence HBC34 wt CDRH3 codon optimized
  source 1..36: mol_type = other DNA
gccgcttggtctggcaacagcggcgggatggatgtc

SEQ ID NO: 75 - DNA, 18 bp, synthetic construct
  misc_feature 1..18: note = Synthetic sequence HBC34 wt CDRL1 codon optimized
  source 1..18: mol_type = other DNA
aaactgggcaacaagaac

SEQ ID NO: 76 - skipped

SEQ ID NO: 77 - DNA, 27 bp, synthetic construct
  misc_feature 1..27: note = Synthetic sequence HBC34 wt CDRL2 long codon optimized
  source 1..27: mol_type = other DNA
gtcatctacgaggtcaagtatcggcca

SEQ ID NO: 78 - DNA, 27 bp, synthetic construct
  misc_feature 1..27: note = Synthetic sequence HBC34 wt CDRL3 codon optimized
  source 1..27: mol_type = other DNA
cagacttgggattcaactactgtcgtg

SEQ ID NO: 79 - protein, 5 aa, synthetic construct
  REGION 1..5: note = Synthetic linker sequence
GGSGG

SEQ ID NO: 80 - protein, 7 aa, Hepatitis B virus
TGPCRTC

SEQ ID NO: 81 - protein, 7 aa, Hepatitis B virus
GNCTCIP

SEQ ID NO: 82 - protein, 25 aa, Hepatitis B virus
  VARIANT 2: note = Cysteine coupled to acetamidomethyl
  source 1..25: note = discontinuous epitope mimic
  VARIANT 21: note = Cysteine coupled to acetamidomethyl
  VARIANT 24: note = Cysteine coupled to acetamidomethyl
CCIPIPSSWAFGCSTTSTGPCRTCC

SEQ ID NO: 83 - protein, 28 aa, Hepatitis B virus
  VARIANT 4: note = Cys is coupled to acetamidomethyl
  source 1..28: note = discontinuous epitope mimic
  VARIANT 6: note = Cys is coupled to acetamidomethyl
  VARIANT 24: note = Cys is coupled to acetamidomethyl
  VARIANT 27: note = Cys is coupled to acetamidomethyl
CGNCTCIPIPSSWAFCSTTSTGPCRTCC

SEQ ID NO: 84 - protein, 17 aa, Hepatitis B virus
  VARIANT 13: note = cys is coupled to acetamidomethyl
  source 1..17: note = looped epitope mimic
  VARIANT 16: note = cys is coupled to acetamidomethyl
CGGGCSTTSTGPCRTCC

SEQ ID NO: 85 - protein, 11 aa, Hepatitis B virus
STTSTGPCRTC

SEQ ID NO: 86 - protein, 15 aa, Hepatitis B virus
GNCTCIPIPSSWAFC

SEQ ID NO: 87 - protein, 14 aa, Hepatitis B virus
GNCTCIPIPSSWAF

SEQ ID NO: 88 - protein, 5 aa, Hepatitis B virus
PCRXC

SEQ ID NO: 89 - protein, 106 aa, synthetic construct
  REGION 1..106: note = Synthetic sequence HBC34-V35 VL
SYELTQPPSVSVSPGQTVSIPCSGDKLGNKNVAWFQHKPGQSPVLVIYEVKYRPSGIPERFSGSNSGNTATLTISGTQAMDEAAYFCQTFDSTTVVFGGGTRLTVL

SEQ ID NO: 90 - protein, 106 aa, synthetic construct
  REGION 1..106: note = Synthetic sequence HBC34-V34 VL
SYELTQPPSVSVSPGQTVSIPCSGDKLGNKNVSWFQHKPGQSPVLVIYEVKYRPSGIPERFSGSNSGNTATLTISGTQAMDEAAYFCQTFDSTTVVFGGGTRLTVL

SEQ ID NO: 91 - protein, 449 aa, synthetic construct
  REGION 1..449: note = Synthetic sequence HC of HBC34-V35-MLNS-GAALIE and HBC34-V34-MLNS-GAALIE (g1M17, 1)
ELQLVESGGGWVQPGGSQRLSCAASGRIFRSFYMSWVRQAPGKGLEWVATINQDGSEKLYVDSVKGRFTISRDNAKNSLFLQMNNLRVEDTAVYYCAAWSGNSGGMDVWGQGTTVSVSSASTKGPSVFPLAPSSKSTSGGTAALGCLVKDYFPEPVTVSWNSGALTSGVHTFPAVLQSSGLYSLSSVVTVPSSSLGTQTYICNVNHKPSNTKVDKKVEPKSCDKTHTCPPCPAPELLAGPSVFLFPPKPKDTLMISRTPEVTCVVVDVSHEDPEVKFNWYVDGVEVHNAKTKPREEQYNSTYRVVSVLTVLHQDWLNGKEYKCKVSNKALPLPEEKTISKAKGQPREPQVYTLPPSRDELTKNQVSLTCLVKGFYPSDIAVEWESNGQPENNYKTTPPVLDSDGSFFLYSKLTVDKSRWQQGNVFSCSVLHEALHSHYTQKSLSLSPGK

SEQ ID NO: 92 - protein, 449 aa, synthetic construct
  REGION 1..449: note = Synthetic sequence HC of HBC34-V35-MLNS and HBC34-V34-MLNS (g1M17, 1)
ELQLVESGGGWVQPGGSQRLSCAASGRIFRSFYMSWVRQAPGKGLEWVATINQDGSEKLYVDSVKGRFTISRDNAKNSLFLQMNNLRVEDTAVYYCAAWSGNSGGMDVWGQGTTVSVSSASTKGPSVFPLAPSSKSTSGGTAALGCLVKDYFPEPVTVSWNSGALTSGVHTFPAVLQSSGLYSLSSVVTVPSSSLGTQTYICNVNHKPSNTKVDKKVEPKSCDKTHTCPPCPAPELLGGPSVFLFPPKPKDTLMISRTPEVTCVVVDVSHEDPEVKFNWYVDGVEVHNAKTKPREEQYNSTYRVVSVLTVLHQDWLNGKEYKCKVSNKALPAPIEKTISKAKGQPREPQVYTLPPSRDELTKNQVSLTCLVKGFYPSDIAVEWESNGQPENNYKTTPPVLDSDGSFFLYSKLTVDKSRWQQGNVFSCSVLHEALHSHYTQKSLSLSPGK

SEQ ID NO: 93 - protein, 212 aa, synthetic construct
  REGION 1..212: note = Synthetic sequence LC of HBC34-V35
SYELTQPPSVSVSPGQTVSIPCSGDKLGNKNVAWFQHKPGQSPVLVIYEVKYRPSGIPERFSGSNSGNTATLTISGTQAMDEAAYFCQTFDSTTVVFGGGTRLTVLGQPKAAPSVTLFPPSSEELQANKATLVCLISDFYPGAVTVAWKADSSPVKAGVETTTPSKQSNNKYAASSYLSLTPEQWKSHRSYSCQVTHEGSTVEKTVAPTECS

SEQ ID NO: 94 - protein, 212 aa, synthetic construct
  REGION 1..212: note = Synthetic sequence LC of HBC34-V34
SYELTQPPSVSVSPGQTVSIPCSGDKLGNKNVSWFQHKPGQSPVLVIYEVKYRPSGIPERFSGSNSGNTATLTISGTQAMDEAAYFCQTFDSTTVVFGGGTRLTVLGQPKAAPSVTLFPPSSEELQANKATLVCLISDFYPGAVTVAWKADSSPVKAGVETTTPSKQSNNKYAASSYLSLTPEQWKSHRSYSCQVTHEGSTVEKTVAPTECS

SEQ ID NO: 95 - protein, 128 aa, synthetic construct
  REGION 1..128: note = Synthetic sequence HBC24 VH
EVQLLESGGGLVQPGGSLRLSCAASGSTFTKYAMSWVRQAPGKGLEWVASISGSVPGFGIDTYYADSVKGRFTISRDTSKNTLYLQMNSLRAEDTALYYCAKDVGVIGSYYYYAMDVWGQGTAVTVSS

SEQ ID NO: 96 - protein, 109 aa, synthetic construct
  REGION 1..109: note = Synthetic sequence HBC24 VL
EIVLTQSPGTLSLSPGERATLSCRASQGLSSSYLAWYQQKPGQAPRLLIYSASTRATGIPDRFSGSGSGTDFTLTISRLEPEDFAVYYCQQYAYSPRWTFGQGTKVEIK

SEQ ID NO: 97 - protein, 8 aa, synthetic construct
  REGION 1..8: note = Synthetic sequence CDRH1 of HBC24
GSTFTKYA

SEQ ID NO: 98 - protein, 8 aa, synthetic construct
  REGION 1..8: note = Synthetic sequence CDRH2 of HBC24
ISGSVPGF

SEQ ID NO: 99 - protein, 21 aa, synthetic construct
  REGION 1..21: note = Synthetic sequence CDRH3 of HBC24
LYYCAKDVGVIGSYYYYAMDV

SEQ ID NO: 100 - protein, 7 aa, synthetic construct
  REGION 1..7: note = Synthetic sequence CDRL1 of HBC24
QGLSSSY

SEQ ID NO: 101 - skipped

SEQ ID NO: 102 - protein, 10 aa, synthetic construct
  REGION 1..10: note = Synthetic sequence CDRL3 of HBC24
QQYAYSPRWT

SEQ ID NO: 103 - DNA, 357 bp, synthetic construct
  misc_feature 1..357: note = Synthetic sequence VH of HBC34-V7, HBC34-V35, and HBC34-V34 (codon optimized)
  source 1..357: mol_type = other DNA
gagctgcagctggtggagtccggcggcggctgggtgcagcctggcggctcccagaggctgagctgtgccgcttctggcaggatcttccggtccttttacatgtcttgggtgcggcaggctccaggcaagggcctggagtgggtggctaccatcaaccaggacggctccgagaagctgtatgtggatagcgtgaagggcagattcacaatctctcgcgacaacgccaagaactccctgtttctgcagatgaacaatctgagggtggaggataccgccgtgtactattgcgccgcttggtctggcaatagcggcggcatggacgtgtggggacagggcaccaccgtgtccgtgtccagc

SEQ ID NO: 104 - DNA, 318 bp, synthetic construct
  misc_feature 1..318: note = Synthetic sequence HBC34-V34 VL (codon optimized)
  source 1..318: mol_type = other DNA
agctacgagctgacacagcccccttccgtgtccgtgtcccctggacagaccgtgtccatcccatgcagcggcgacaagctgggcaacaagaacgtgtcctggtttcagcataagcctggccagtcccccgtgctggtcatctacgaggtgaagtataggcccagcggcatccctgagcggttctctggctccaacagcggcaatacagccaccctgacaatctctggcacacaggctatggacgaggccgcttatttctgccagacctttgattccaccacagtggtgttcggcggcggcaccagactgacagtgctg

SEQ ID NO: 105 - DNA, 318 bp, synthetic construct
  misc_feature 1..318: note = Synthetic sequence HBC34-V35 VL (codon optimized)
  source 1..318: mol_type = other DNA
agctacgagctgacacagcccccttccgtgtccgtgtcccctggacagaccgtgtccatcccatgcagcggcgacaagctgggcaacaagaacgtggcctggtttcagcataagcctggccagtcccccgtgctggtcatctacgaggtgaagtataggcccagcggcatccctgagcggttctctggctccaacagcggcaatacagccaccctgacaatctctggcacacaggctatggacgaggccgcttatttctgccagacctttgattccaccacagtggtgttcggcggcggcaccagactgacagtgctg

SEQ ID NO: 106 - DNA, 360 bp, synthetic construct
  misc_feature 1..360: note = Synthetic sequence HBC24 VH (wild type)
  source 1..360: mol_type = other DNA
gaggtgcagttgttggagtctgggggaggcttggtacagcctggggggtccctgagactctcctgtgcagcctctggatccacttttaccaaatatgccatgagctgggtccgtcaggctccagggaaggggctggagtgggtcgcaagtattagtggaagtgttcctggttttggtattgacacatactacgcagactccgttaagggccggttcaccatctccagagacacttccaagaacaccctgtatctgcaaatgaacagcctgagagccgaggacacggccttatattactgtgcgaaagatgtcggggttatcgggtcatactattactacgctatggacgtctggggtcaa

SEQ ID NO: 107 - DNA, 327 bp, synthetic construct
  misc_feature 1..327: note = Synthetic sequence HBC24 VL (wild type)
  source 1..327: mol_type = other DNA
aaattgtgttgacgcagtctccaggcaccctgtctttgtctccaggggaaagagccaccctctcctgcagggccagtcagggtcttagcagcagttacttagcctggtaccagcagaaacctggccaggctcccaggctcctcatctatagtgcgtccaccagggccactggcatcccagacaggttcagtggcagtgggtctgggacagacttcactctcaccatcagcagactggagcctgaagattttgcagtgtattactgtcaacagtatgcttactcacctcggtggacgttcggccaagggaccaaggtggagatcaaac

SEQ ID NO: 108 - DNA, 384 bp, synthetic construct
  misc_feature 1..384: note = Synthetic sequence HBC24 VH (codon optimized)
  source 1..384: mol_type = other DNA
gaggtgcagctgctggaaagcggcggcggcctggtgcagcccggcggctccctgaggctgtcttgcgccgcctctggcagcaccttcacaaagtatgcaatgtcttgggtgcgccaggcaccaggcaagggcctggagtgggtggcctccatctctggcagcgtgcctggcttcggcatcgacacctactatgccgattccgtgaagggccggtttacaatcagcagagacacctccaagaacacactgtatctgcagatgaattctctgcgggccgaggacaccgccctgtactattgtgccaaggatgtgggcgtgatcggcagctactattactatgcaatggacgtgtggggacagggaacagcagtgacagtgagctcc

SEQ ID NO: 109 - DNA, 327 bp, synthetic construct
  misc_feature 1..327: note = Synthetic sequence HBC24 VL (codon optimized)
  source 1..327: mol_type = other DNA
gagatcgtgctgacccagtctcctggcacactgtccctgtcccctggagagagagccaccctgtcctgcagagcctctcagggcctgagctcctcttacctggcctggtatcagcagaagcctggacaggcccctcggctgctgatctactctgcctccaccagagcaacaggcattcctgaccgcttctccggatctggaagcggcacagacttcaccctgacaatcagccggctggagcctgaggacttcgccgtgtactattgtcagcagtacgcctattccccaaggtggacctttggccagggcacaaaggtggagatcaag

SEQ ID NO: 110 - DNA, 318 bp, synthetic construct
  misc_feature 1..318: note = Synthetic sequence HBC34-V7 VL (codon optimized)
  source 1..318: mol_type = other DNA
agctacgagctgacacagcccccttccgtgtccgtgtcccctggacagaccgtgtccatcccatgcagcggcgacaagctgggcaacaagaacgtgtgctggtttcagcataagcctggccagtcccccgtgctggtcatctacgaggtgaagtataggcccagcggcatccctgagcggttctctggctccaacagcggcaatacagccaccctgacaatctctggcacacaggctatggacgaggccgcttatttctgccagacctttgattccaccacagtggtgttcggcggcggcaccagactgacagtgctg

SEQ ID NO: 111 - protein, 106 aa, synthetic construct
  REGION 1..106: note = Synthetic sequence HBC34v23-L_C40S
SYELTQPPSVSVSPGQTASITCSGDKLGNKNASWYQQKPGQSPVLVIYEVKYRPSGIPERFSGSNSGNTATLTISGTQAMDEADYYCQTFDSTTVVFGGGTKLTVL

SEQ ID NO: 112 - protein, 106 aa, synthetic construct
  REGION 1..106: note = Synthetic sequence HBC34v23-L_C40A
SYELTQPPSVSVSPGQTASITCSGDKLGNKNAAWYQQKPGQSPVLVIYEVKYRPSGIPERFSGSNSGNTATLTISGTQAMDEADYYCQTFDSTTVVFGGGTKLTVL

SEQ ID NO: 113 - protein, 106 aa, synthetic construct
  REGION 1..106: note = Synthetic sequence HBC34v31-L_C40S
SYELTQPPSVSVSPGQTVSIPCSGDKLGNKNVSWFQHKPGQSPVLVIYEVKYRPSGIPERFSGSNSGNTATLTISGTQAMDEAAYFCQTWDSTTVVFGGGTRLTVL

SEQ ID NO: 114 - protein, 106 aa, synthetic construct
  REGION 1..106: note = Synthetic sequence HBC34v31-L_C40A
SYELTQPPSVSVSPGQTVSIPCSGDKLGNKNVAWFQHKPGQSPVLVIYEVKYRPSGIPERFSGSNSGNTATLTISGTQAMDEAAYFCQTWDSTTVVFGGGTRLTVL

SEQ ID NO: 115 - protein, 106 aa, synthetic construct; identical to SEQ ID NO: 90
  REGION 1..106: note = Synthetic sequence HBC34v32-L_C40S

SEQ ID NO: 116 - protein, 106 aa, synthetic construct; identical to SEQ ID NO: 114
  REGION 1..106: note = Synthetic sequence HBC34v32-L_C40A

SEQ ID NO: 117 - protein, 106 aa, synthetic construct; identical to SEQ ID NO: 111
  REGION 1..106: note = Synthetic sequence HBC34v33-L_C40S

SEQ ID NO: 118 - protein, 106 aa, synthetic construct; identical to SEQ ID NO: 112
  REGION 1..106: note = Synthetic sequence HBC34v33-L_C40A

SEQ ID NO: 119 - protein, 106 aa, synthetic construct; identical to SEQ ID NO: 113
  REGION 1..106: note = Synthetic sequence HBC34-L_C40S

SEQ ID NO: 120 - protein, 106 aa, synthetic construct; identical to SEQ ID NO: 114
  REGION 1..106: note = Synthetic sequence HBC34-L_C40A

SEQ ID NO: 121 - protein, 458 aa, synthetic construct
  REGION 1..458: note = Synthetic sequence HBC24-MLNS
EVQLLESGGGLVQPGGSLRLSCAASGSTFTKYAMSWVRQAPGKGLEWVASISGSVPGFGIDTYYADSVKGRFTISRDTSKNTLYLQMNSLRAEDTALYYCAKDVGVIGSYYYYAMDVWGQGTAVTVSSASTKGPSVFPLAPSSKSTSGGTAALGCLVKDYFPEPVTVSWNSGALTSGVHTFPAVLQSSGLYSLSSVVTVPSSSLGTQTYICNVNHKPSNTKVDKKVEPKSCDKTHTCPPCPAPELLGGPSVFLFPPKPKDTLMISRTPEVTCVVVDVSHEDPEVKFNWYVDGVEVHNAKTKPREEQYNSTYRVVSVLTVLHQDWLNGKEYKCKVSNKALPAPIEKTISKAKGQPREPQVYTLPPSRDELTKNQVSLTCLVKGFYPSDIAVEWESNGQPENNYKTTPPVLDSDGSFFLYSKLTVDKSRWQQGNVFSCSVLHEALHSHYTQKSLSLSPGK

SEQ ID NO: 122 - protein, 458 aa, synthetic construct
  REGION 1..458: note = Synthetic sequence HBC24-MLNS-GAALIE
EVQLLESGGGLVQPGGSLRLSCAASGSTFTKYAMSWVRQAPGKGLEWVASISGSVPGFGIDTYYADSVKGRFTISRDTSKNTLYLQMNSLRAEDTALYYCAKDVGVIGSYYYYAMDVWGQGTAVTVSSASTKGPSVFPLAPSSKSTSGGTAALGCLVKDYFPEPVTVSWNSGALTSGVHTFPAVLQSSGLYSLSSVVTVPSSSLGTQTYICNVNHKPSNTKVDKKVEPKSCDKTHTCPPCPAPELLAGPSVFLFPPKPKDTLMISRTPEVTCVVVDVSHEDPEVKFNWYVDGVEVHNAKTKPREEQYNSTYRVVSVLTVLHQDWLNGKEYKCKVSNKALPLPEEKTISKAKGQPREPQVYTLPPSRDELTKNQVSLTCLVKGFYPSDIAVEWESNGQPENNYKTTPPVLDSDGSFFLYSKLTVDKSRWQQGNVFSCSVLHEALHSHYTQKSLSLSPGK

SEQ ID NO: 123 - protein, 449 aa, synthetic construct
  REGION 1..449: note = Synthetic sequence HBC34-V7-mu (IgG2a) HC
ELQLVESGGGWVQPGGSQRLSCAASGRIFRSFYMSWVRQAPGKGLEWVATINQDGSEKLYVDSVKGRFTISRDNAKNSLFLQMNNLRVEDTAVYYCAAWSGNSGGMDVWGQGTTVSVSSAKTTAPSVYPLAPVCGDTTGSSVTLGCLVKGYFPEPVTLTWNSGSLSSGVHTFPAVLQSDLYTLSSSVTVTSSTWPSQSITCNVAHPASSTKVDKKIEPRGPTIKPCPPCKCPAPNLLGGPSVFIFPPKIKDVLMISLSPIVTCVVVDVSEDDPDVQISWFVNNVEVHTAQTQTHREDYNSTLRVVSALPIQHQDWMSGKEFKCKVNNKDLPAPIERTISKPKGSVRAPQVYVLPPPEEEMTKKQVTLTCMVTDFMPEDIYVEWTNNGKTELNYKNTEPVLDSDGSYFMYSKLRVEKKNWVERNSYSCSVVHEGLHNHHTTKSFSRTPGK

SEQ ID NO: 124 - protein, 212 aa, synthetic construct
  REGION 1..212: note = Synthetic sequence HBC34-V7-mu (IgG2a) LC
SYELTQPPSVSVSPGQTVSIPCSGDKLGNKNVCWFQHKPGQSPVLVIYEVKYRPSGIPERFSGSNSGNTATLTISGTQAMDEAAYFCQTFDSTTVVFGGGTRLTVLGQPKSSPSVTLFPPSSEELETNKATLVCTITDFYPGVVTVDWKVDGTPVTQGMETTQPSKQSNNKYMASSYLTLTARAWERHSSYSCQVTHEGHTVEKSLSRADCS

SEQ ID NO: 125 - protein, 449 aa, synthetic construct; identical to SEQ ID NO: 123
  REGION 1..449: note = Synthetic sequence HBC34-V35-mu (IgG2a) HC

SEQ ID NO: 126 - protein, 212 aa, synthetic construct
  REGION 1..212: note = Synthetic sequence HBC34-V35-mu (IgG2a) LC
SYELTQPPSVSVSPGQTVSIPCSGDKLGNKNVAWFQHKPGQSPVLVIYEVKYRPSGIPERFSGSNSGNTATLTISGTQAMDEAAYFCQTFDSTTVVFGGGTRLTVLGQPKSSPSVTLFPPSSEELETNKATLVCTITDFYPGVVTVDWKVDGTPVTQGMETTQPSKQSNNKYMASSYLTLTARAWERHSSYSCQVTHEGHTVEKSLSRADCS

SEQ ID NO: 127 - protein, 458 aa, synthetic construct
  REGION 1..458: note = Synthetic sequence HBC24-mu (IgG2a) HC
EVQLLESGGGLVQPGGSLRLSCAASGSTFTKYAMSWVRQAPGKGLEWVASISGSVPGFGIDTYYADSVKGRFTISRDTSKNTLYLQMNSLRAEDTALYYCAKDVGVIGSYYYYAMDVWGQGTAVTVSSAKTTAPSVYPLAPVCGDTTGSSVTLGCLVKGYFPEPVTLTWNSGSLSSGVHTFPAVLQSDLYTLSSSVTVTSSTWPSQSITCNVAHPASSTKVDKKIEPRGPTIKPCPPCKCPAPNLLGGPSVFIFPPKIKDVLMISLSPIVTCVVVDVSEDDPDVQISWFVNNVEVHTAQTQTHREDYNSTLRVVSALPIQHQDWMSGKEFKCKVNNKDLPAPIERTISKPKGSVRAPQVYVLPPPEEEMTKKQVTLTCMVTDFMPEDIYVEWTNNGKTELNYKNTEPVLDSDGSYFMYSKLRVEKKNWVERNSYSCSVVHEGLHNHHTTKSFSRTPGK

SEQ ID NO: 128 - protein, 215 aa, synthetic construct
  REGION 1..215: note = Synthetic sequence HBC24-mu (IgG2a) LC
EIVLTQSPGTLSLSPGERATLSCRASQGLSSSYLAWYQQKPGQAPRLLIYSASTRATGIPDRFSGSGSGTDFTLTISRLEPEDFAVYYCQQYAYSPRWTFGQGTKVEIKADAAPTVSIFPPSSEQLTSGGASVVCFLNNFYPKDINVKWKIDGSERQNGVLNSWTDQDSKDSTYSMSSTLTLTKDEYERHNSYTCEATHKTSTSPIVKSFNRNEC

SEQ ID NO: 129 - protein, 449 aa, synthetic construct
  REGION 1..449: note = Synthetic sequence HBC34-V7, HBC34-V34, HBC34-V35 HC (wild-type)
ELQLVESGGGWVQPGGSQRLSCAASGRIFRSFYMSWVRQAPGKGLEWVATINQDGSEKLYVDSVKGRFTISRDNAKNSLFLQMNNLRVEDTAVYYCAAWSGNSGGMDVWGQGTTVSVSSASTKGPSVFPLAPSSKSTSGGTAALGCLVKDYFPEPVTVSWNSGALTSGVHTFPAVLQSSGLYSLSSVVTVPSSSLGTQTYICNVNHKPSNTKVDKKVEPKSCDKTHTCPPCPAPELLGGPSVFLFPPKPKDTLMISRTPEVTCVVVDVSHEDPEVKFNWYVDGVEVHNAKTKPREEQYNSTYRVVSVLTVLHQDWLNGKEYKCKVSNKALPAPIEKTISKAKGQPREPQVYTLPPSRDELTKNQVSLTCLVKGFYPSDIAVEWESNGQPENNYKTTPPVLDSDGSFFLYSKLTVDKSRWQQGNVFSCSVMHEALHNHYTQKSLSLSPGK

SEQ ID NO: 130 - DNA, 990 bp, synthetic construct
  misc_feature 1..990: note = Synthetic sequence HBC34-V7, HBC34-V34, HBC34-V35 CH1-hinge-CH2-CH3 (codon-optimized)
  source 1..990: mol_type = other DNA
gcctccacaaagggcccaagcgtgtttccactggctccctcttccaagtctacctccggcggcacagccgctctgggatgtctggtgaaggattacttcccagagcccgtgaccgtgtcttggaactccggcgccctgaccagcggagtgcatacatttccagctgtgctgcagagctctggcctgtactctctgtccagcgtggtgaccgtgccctcttccagcctgggcacccagacatatatctgcaacgtgaatcacaagccaagcaatacaaaggtggacaagaaggtggagcccaagtcttgtgataagacccatacatgccctccatgtccagctccagagctgctgggcggcccaagcgtgttcctgtttccacccaagcctaaggataccctgatgatctccagaacccccgaggtgacatgcgtggtggtggacgtgagccacgaggatcctgaggtgaagttcaactggtacgtggacggcgtggaggtgcataatgctaagaccaagcccagggaggagcagtacaactctacctatcgggtggtgtccgtgctgacagtgctgcaccaggattggctgaacggcaaggagtataagtgcaaggtgtctaataaggccctgcccgctcctatcgagaagaccatctccaaggccaagggccagcctagagagccacaggtgtacacactgcctccatctcgcgatgagctgaccaagaaccaggtgtccctgacatgtctggtgaagggcttctatccttccgacatcgctgtggagtgggagagcaatggccagccagagaacaattacaagaccacaccccctgtgctggacagcgatggctctttctttctgtatagcaagctgaccgtggacaagtctcgctggcagcagggcaacgtgtttagctgttctgtgatgcatgaggccctgcacaatcattatacacagaagtccctgagcctgtctcctggcaag

SEQ ID NO: 131 - DNA, 1417 bp, synthetic construct
  misc_feature 1..1417: note = Synthetic sequence HBC34-V7, HBC34-V34, HBC34-V35 VH-CH1-hinge-CH2-CH3 (codon-optimized)
  source 1..1417: mol_type = other DNA
gagctgcagctggtggagtccggcggcggctgggtgcagcctggcggctcccagaggctgagctgtgccgcttctggcaggatcttccggtccttttacatgtcttgggtgcggcaggctccaggcaagggcctggagtgggtggctaccatcaaccaggacggctccgagaagctgtatgtggatagcgtgaagggcagattcacaatctctcgcgacaacgccaagaactccctgtttctgcagatgaacaatctgagggtggaggataccgccgtgtactattgcgccgcttggtctggcaatagcggcggcatggacgtgtggggacagggcaccaccgtgtccgtgtccagcgcctccacaaagggcccaagcgtgtttccactggctccctcttccaagtctacctccggcggcacagccgctctgggatgtctggtgaaggattacttcccagagcccgtgaccgtgtcttggaactccggcgccctgaccagcggagtgcatacatttccagctgtgctgcagagctctggcctgtactctctgtccagcgtggtgaccgtgccctcttccagcctgggcacccagacatatatctgcaacgtgaatcacaagccaagcaatacaaaggtggacaagaaggtggagcccaagtcttgtgataagacccatacatgccctccatgtccagctccagagctgctgggcggcccaagcgtgttcctgtttccacccaagcctaaggataccctgatgatctccagaacccccgaggtgacatgcgtggtggtggacgtgagccacgaggatcctgaggtgaagttcaactggtacgtggacggcgtggaggtgcataatgctaagaccaagcccagggaggagcagtacaactctacctatcgggtggtgtccgtgctgacagtgctgcaccaggattggctgaacggcaaggagtataagtgcaaggtgtctaataaggccctgcccgctcctatcgagaagaccatctccaaggccaagggccagcctagagagccacaggtgtacacactgcctccatctcgcgatgagctgaccaagaaccaggtgtccctgacatgtctggtgaagggcttctatccttccgacatcgctgtggagtgggagagcaatggccagccagagaacaattacaagaccacaccccctgtgctggacagcgatggctctttctttctgtatagcaagctgaccgtggacaagtctcgctggcagcagggcaacgtgtttagctgttctgtgatgcatgaggccctgcacaatcattatacacagaagtccctgagcctgtctcctggcaagtgatgaggtaccgtgcgacggccggcaagcccccgctccccgggctctcgcggtcgtacgaggaaagctt

SEQ ID NO: 132 - DNA, 318 bp, synthetic construct
  misc_feature 1..318: note = Synthetic sequence HBC34-V7 CL (codon-optimized)
  source 1..318: mol_type = other DNA
ggacagccaaaggctgctccatctgtgaccctgtttccaccctcttccgaggagctgcaggccaacaaggccaccctggtgtgcctgatctctgacttctaccctggagctgtgacagtggcttggaaggctgatagctctcccgtgaaggctggcgtggagacaacaacccctagcaagcagtctaacaataagtacgccgcttccagctatctgtctctgacaccagagcagtggaagtcccaccgctcttattcctgccaggtgacccatgagggcagcaccgtggagaagacagtggcccccaccgagtgttct

SEQ ID NO: 133 - DNA, 636 bp, synthetic construct
  misc_feature 1..636: note = Synthetic sequence HBC34-V7 LC (VL-CL) (codon-optimized)
  source 1..636: mol_type = other DNA
agctacgagctgacacagcccccttccgtgtccgtgtcccctggacagaccgtgtccatcccatgcagcggcgacaagctgggcaacaagaacgtgtgctggtttcagcataagcctggccagtcccccgtgctggtcatctacgaggtgaagtataggcccagcggcatccctgagcggttctctggctccaacagcggcaatacagccaccctgacaatctctggcacacaggctatggacgaggccgcttatttctgccagacctttgattccaccacagtggtgttcggcggcggcaccagactgacagtgctgggacagccaaaggctgctccatctgtgaccctgtttccaccctcttccgaggagctgcaggccaacaaggccaccctggtgtgcctgatctctgacttctaccctggagctgtgacagtggcttggaaggctgatagctctcccgtgaaggctggcgtggagacaacaacccctagcaagcagtctaacaataagtacgccgcttccagctatctgtctctgacaccagagcagtggaagtcccaccgctcttattcctgccaggtgacccatgagggcagcaccgtggagaagacagtggcccccaccgagtgttct

SEQ ID NO: 134 - DNA, 318 bp, synthetic construct; identical to SEQ ID NO: 132
  misc_feature 1..318: note = Synthetic sequence HBC34-V34, HBC34-V35 CL (codon-optimized)
  source 1..318: mol_type = other DNA

SEQ ID NO: 135 - DNA, 636 bp, synthetic construct
  misc_feature 1..636: note = Synthetic sequence HBC34-V34 LC (VL-CL) (codon-optimized)
  source 1..636: mol_type = other DNA
agctacgagctgacacagcccccttccgtgtccgtgtcccctggacagaccgtgtccatcccatgcagcggcgacaagctgggcaacaagaacgtgtcctggtttcagcataagcctggccagtcccccgtgctggtcatctacgaggtgaagtataggcccagcggcatccctgagcggttctctggctccaacagcggcaatacagccaccctgacaatctctggcacacaggctatggacgaggccgcttatttctgccagacctttgattccaccacagtggtgttcggcggcggcaccagactgacagtgctgggacagccaaaggctgctccatctgtgaccctgtttccaccctcttccgaggagctgcaggccaacaaggccaccctggtgtgcctgatctctgacttctaccctggagctgtgacagtggcttggaaggctgatagctctcccgtgaaggctggcgtggagacaacaacccctagcaagcagtctaacaataagtacgccgcttccagctatctgtctctgacaccagagcagtggaagtcccaccgctcttattcctgccaggtgacccatgagggcagcaccgtggagaagacagtggcccccaccgagtgttct

SEQ ID NO: 136 - DNA, 636 bp, synthetic construct
  misc_feature 1..636: note = Synthetic sequence HBC34-V35 LC (VL-CL) (codon-optimized)
  source 1..636: mol_type = other DNA
agctacgagctgacacagcccccttccgtgtccgtgtcccctggacagaccgtgtccatcccatgcagcggcgacaagctgggcaacaagaacgtggcctggtttcagcataagcctggccagtcccccgtgctggtcatctacgaggtgaagtataggcccagcggcatccctgagcggttctctggctccaacagcggcaatacagccaccctgacaatctctggcacacaggctatggacgaggccgcttatttctgccagacctttgattccaccacagtggtgttcggcggcggcaccagactgacagtgctgggacagccaaaggctgctccatctgtgaccctgtttccaccctcttccgaggagctgcaggccaacaaggccaccctggtgtgcctgatctctgacttctaccctggagctgtgacagtggcttggaaggctgatagctctcccgtgaaggctggcgtggagacaacaacccctagcaagcagtctaacaataagtacgccgcttccagctatctgtctctgacaccagagcagtggaagtcccaccgctcttattcctgccaggtgacccatgagggcagcaccgtggagaagacagtggcccccaccgagtgttct

SEQ ID NO: 137 - protein, 217 aa, Homo sapiens
  REGION 1..217: note = WT hIgG1 Fc
APELLGGPSVFLFPPKPKDTLMISRTPEVTCVVVDVSHEDPEVKFNWYVDGVEVHNAKTKPREEQYNSTYRVVSVLTVLHQDWLNGKEYKCKVSNKALPAPIEKTISKAKGQPREPQVYTLPPSRDELTKNQVSLTCLVKGFYPSDIAVEWESNGQPENNYKTTPPVLDSDGSFFLYSKLTVDKSRWQQGNVFSCSVMHEALHNHYTQKSLSLSPGK

SEQ ID NO: 138 - protein, 449 aa, synthetic construct
  REGION 1..449: note = Synthetic sequence HBC34, HBC34v7, HBC34v23, HBC34v34, HBC34v35, HBC34_C40S, HBC34_C40A, HBC34v23_C40S, HBC34v23_C40A HC with GAALIE mutation in hIgG1 Fc
ELQLVESGGGWVQPGGSQRLSCAASGRIFRSFYMSWVRQAPGKGLEWVATINQDGSEKLYVDSVKGRFTISRDNAKNSLFLQMNNLRVEDTAVYYCAAWSGNSGGMDVWGQGTTVSVSSASTKGPSVFPLAPSSKSTSGGTAALGCLVKDYFPEPVTVSWNSGALTSGVHTFPAVLQSSGLYSLSSVVTVPSSSLGTQTYICNVNHKPSNTKVDKKVEPKSCDKTHTCPPCPAPELLAGPSVFLFPPKPKDTLMISRTPEVTCVVVDVSHEDPEVKFNWYVDGVEVHNAKTKPREEQYNSTYRVVSVLTVLHQDWLNGKEYKCKVSNKALPLPEEKTISKAKGQPREPQVYTLPPSRDELTKNQVSLTCLVKGFYPSDIAVEWESNGQPENNYKTTPPVLDSDGSFFLYSKLTVDKSRWQQGNVFSCSVMHEALHNHYTQKSLSLSPGK

SEQ ID NO: 139 - protein, 19 aa, synthetic construct
  REGION 1..19: note = Chimeric hinge sequence
ESKYGPPCPPCPAPPVAGP